European Patent Specification EP 4 231 962 B1, published April 9, 2025. Title: Beschichtetes Haar und dessen Verwendung. Applicant: Strauch, Georg. The sequence listing filed with the application follows.

SEQUENCE LISTING (13 sequences)

SEQ ID NO: 1 - protein, 5 aa, Artificial Sequence
  Wiederholungssequenz aus Seidenprotein
  Xaa (4)..(5): jedes Xaa kann unabhängig voneinander jede beliebige natürliche Aminosäure sein
GPGXX

SEQ ID NO: 2 - protein, 5 aa, Artificial Sequence
  Wiederholungssequenz aus Seidenprotein
  Xaa (5)..(5): Xaa kann jede beliebige natürliche Aminosäure sein
GVPGX

SEQ ID NO: 3 - protein, 5 aa, Artificial Sequence
  Wiederholungssequenz aus Seidenprotein
  Xaa (4)..(5): jedes Xaa kann unabhängig voneinander jede beliebige natürliche Aminosäure sein
GSGXX

SEQ ID NO: 4 - protein, 5 aa, Artificial Sequence
  Wiederholungssequenz aus Seidenprotein
  Xaa (4)..(5): jedes Xaa kann unabhängig voneinander jede beliebige natürliche Aminosäure sein
GGYXX

SEQ ID NO: 5 - protein, 5 aa, Artificial Sequence
  Wiederholungssequenz aus Seidenprotein
  Xaa (4)..(5): jedes Xaa kann unabhängig voneinander jede beliebige natürliche Aminosäure sein
PQQXX

SEQ ID NO: 6 - protein, 5 aa, Artificial Sequence
  Wiederholungssequenz aus Seidenprotein
  Xaa (4)..(5): jedes Xaa kann unabhängig voneinander jede beliebige natürliche Aminosäure sein
GYGXX

SEQ ID NO: 7 - protein, 5263 aa, Bombyx mori
MRVKTFVILCCALQYVAYTNANINDFDEDYFGSDVTVQSSNTTDEIIRDASGAVIEEQITTKKMQRKNKNHGILGKNEKMIKTFVITTDSDGNESIVEEDVLMKTLSDGTVAQSYVAADAGAYSQSGPYVSNSGYSTHQGYTSDFSTSAAVGAGAGAGAAAGSGAGAGAGYGAASGAGAGAGAGAGAGYGTGAGAGAGAGYGAGAGAGAGAGYGAGAGAGAGAGYGAGAGAGAGAGYGAGAGAGAGAGYGAGAGAGAGAGYGAASGAGAGAGYGQGVGSGAASGAGAGAGAGSAAGSGAGAGAGTGAGAGYGAGAGAGAGAGYGAASGTGAGYGAGAGAGYGGASGAGAGAGAGAGAGAGAGYGTGAGYGAGAGAGAGAGAGAGYGAGAGAGYGAGYGVGAGAGYGAGYGAGAGSGAASGAGSGAGAGSGAGAGSGAGAGSGAGAGSGAGAGSGAGAGSGAGAGSGAGAGSGTGAGSGAGAGYGAGAGAGYGAGAGSGAASGAGAGSGAGAGSGAGAGSGAGAGSGAGAGSGAGAGYGAGAGAGYGAGAGAGYGAGAGVGYGAGAGSGAASGAGAGSGAGAGSGAGAGSGAGAGSGAGAGSGAGAGSGAGAGSGAGAGSGAGAGSGAGVGYGAGVGAGYGAGYGAGAGAGYGAGAGSGAASGAGAGAGAGAGTGSSGFGPYVANGGYSRSDGYEYAWSSDFGTGSGAGAGSGAGAGSGAGAGSGAGAGSGAGAGSGAGAGYGAGVGVGYGAGYGAGAGAGYGAGAGSGAASGAGAGSGAGAGSGAGAGSGAGAGSGAGAGSGAGAGSGAGAGSGAGAGSGAGAGSGAGAGSGAGVGSGAGAGSGAGAGVGYGAGAGVGYGAGAGSGAASGAGAGSGAGAGSGAGAGSGAGAGSGAGAGSGAGAGSGAGAGSGAGAGSGAGAGSGAGVGYGAGVGAGYGAGYGAGAGAGYGAGAGSGAASGAGAGSGAGAGSGAGAGSGAGAGSGAGAGSGAGAGSGAGAGSGAGAGSGAGAGSGAGAGSGAGAGSGAGAGYGAGAGAGYGAGYGAGAGAGYGAGAGSGAASGAGSGAGAGSGAGAGAGSGAGAGSGAGAGSGAGAGSGAGAGSGAGAGSGAGAGYGAGVGAGYGAGYGAGAGAGYGAGAGSGAASGAGAGSGAGAGSGAGAGSGAGAGSGAGAGSGAGAGSGAGAGSGAGVGYGAGYGAGAGAGYGAGAGSGAASGAGAGAGAGAGTGSSGFGPYVAHGGYSGYEYAWSSESDFGTGSGAGAGSGAGAGSGAGAGSGAGAGSGAGYGAGVGAGYGAGYGAGAGAGYGAGAGSGAGSGAGAGSGAGAGSGAGAGSGAGAGSGAGAGSGAGAGSGAGAGSGAGAGSGAGAGYGAGYGAGAGAGYGAGAGSGAGSGAGAGSGAGAGSGAGAGSGAGAGSGAGAGSGAGAGSGAGAGSGAGAGYGAGVGAGYGAGYGAGAGAGYGAGAGSGAGSGAGAGSGAGAGSGAGAGSGAGVGSGAGAGSGAGAGSGAGAGSGAGAGYGAGYGAGAGAGYGAGAGSGAGSGAGAGSGAGAGSGAGAGSGAGAGSGAGAGSGAGAGSGAGAGSGAGVGYGAGVGAGYGAGYGAGAGAGYGAGAGSGAASGAGAGAGAGAGTGSSGFGPYVANGGYSGYEYAWSSESDFGTGSGAGAGSGAGAGSGAGAGSGAGAGSGAGAGYGAGYGAGAGAGYGAGAGSGAGSGAGAGSGAGAGSGAGAGSGAGAGSGAGAGSGAGAGSGAGAGSGAGSGSGAGAGSGAGAGSGAGAGYGAGVGAGYGVGYGAGAGAGYGAGAGSGAASGAGAGAGAGAGTGSSGFGPYVAHGGYSGYEYAWSSESDFGTGSGAGAGSGAGAGSGAGAGSGAGAGSGAGAGSGAGAGSGAGAGYGAGVGAGYGAAYGAGAGAGYGAGAGSGAASGAGAGSGAGAGSGAGAGSGAGAGSGAGAGSGAGAGSGAGAGSGAGAGSGAGAGSGAGAGSGAGAGYGAGAGAGYGAGAGSGAGSGAGAGSGAGAGSGAGAGSGAGAGSGAGAGSGAGSGSGAGAGSGAGAGSGAGAGYGAGVGAGYGAGYGAGAGAGYGAGAGSGAGSGAGAGSGAGAGYGAGAGAGYGAGYGAGAGAGYGAGAGTGAGSGAGAGSGAGAGSGAGAGSGAGAGSGAGAGSGAGAGSGAGSGSGAGAGSGAGAGSGAGAGSGAGAGSGAGAGSGAGAGYGAGAGAGYGAGYGAGAGAGYGAGAGSGAGSGAGAGSGAGAGSGAGAGSGAGAGYGAGYGAGAGSGAASGAGAGAGAGAGTGSSGFGPYVAHGGYSGYEYAWSSESDFGTGSGAGAGSGAGAGAGAGAGSGAGAGYGAGVGAGYGAGYGAGAGAGYGAGAGSGTGSGAGAGSGAGAGYGAGVGAGYGAGAGSGAAFGAGAGAGAGSGAGAGSGAGAGSGAGAGSGAGAGSGAGAGYGAGYGAGVGAGYGAGAGSGAASGAGAGSGAGAGSGAGAGSGAGAGSGAGAGSGAGAGYGAGVGAGYGAGYGAGAGAGYGAGAGSGAASGAGAGSGAGAGAGSGAGAGSGAGAGSGAGAGSGAGSGAGAGSGAGAGSGAGAGYGAGAGSGAASGAGAGAGAGAGTGSSGFGPYVANGGYSGYEYAWSSESDFGTGSGAGAGSGAGAGSGAGAGSGAGAGSGAGAGYGAGVGAGYGAGYGAGAGAGYGAGAGSGAGSGAGAGSGAGAGSGAGAGSGAGAGSGAGAGSGAGAGSGAGAGYGAGAGSGAASGAGAGSGAGAGSGAGAGSGAGAGSGAGAGSGAGAGSGAGAGYGAGVGAGYGVGYGAGAGAGYGAGAGSGAGSGAGAGSGAGAGSGAGAGSGAGAGSGAGSGAGAGSGAGAGSGAGAGSGAGSGAGAGSGAGAGYGVGYGAGAGAGYGAGAGSGAGSGAGAGSGAGAGSGAGAGSGAGSGAGAGSGAGAGSGAGAGSGAGAGYGAGVGAGYGVGYGAGAGAGYGAGAGSGAGSGAGAGSGAGAGSGAGAGSGAGAGSGAGAGSGAGAGSGAGAGSGAGSGAGAGSGAGAGSGAGAGSGAGAGSGAGSGAGAGSGAGAGSGAGAGSGAGAGYGAGVGAGYGVGYGAGVGAGYGAGAGSGAASGAGAGSGAGAGAGSGAGAGSGAGAGSGAGAGSGAGAGSGAGAGSGAGAGYGAGYGAGVGAGYGAGAGVGYGAGAGAGYGAGAGSGAASGAGAGAGSGAGAGTGAGAGSGAGAGYGAGAGSGAASGAGAGAGAGAGTGSSGFGPYVANGGYSGYEYAWSSESDFGTGSGAGAGSGAGAGSGAGAGSGAGAGSGAGAGYGAGVGAGYGAGAGSGAGSGAGAGSGAGAGSGAGAGSGAGAGSGAGAGYGAGAGSGTGSGAGAGSGAGAGSGAGAGSGAGAGSGAGAGSGAGAGSGVGAGYGVGYGAGAGAGYGVGYGAGAGAGYGAGAGSGTGSGAGAGSGAGAGSGAGAGSGAGAGSGAGAGSGAGAGSGAGAGYGAGVGAGYGVGYGAGAGAGYGAGAGSGAGSGAGAGSGAGAGSGAGAGSGAGAGSGAGSGAGAGSGAGAGSGAGAGSGAGSGAGAGSGAGAGYGVGYGAGAGAGYGAGAGSGAGSGAGAGSGAGAGSGAGAGSGAGSGAGAGSGAGAGSGAGAGSGAGAGYGAGVGAGYGVGYGAGAGAGYGAGAGSGAGSGAGAGSGAGAGSGAGAGSGAGAGSGAGAGSGAGAGSGAGAGSGAGSGAGAGSGAGAGSGAGAGSGAGAGYGAGVGAGYGVGYGAGAGAGYGAGAGSGAASGAGAGAGAGAGTGSSGFGPYVANGGYSGYEYAWSSESDFGTGSGAGAGSGAGAGSGAGAGYGAGYGAGVGAGYGAGAGVGYGAGAGAGYGAGAGSGAASGAGAGAGAGAGSGAGAGSGAGAGAGSGAGAGYGAGYGIGVGAGYGAGAGVGYGAGAGAGYGAGAGSGAASGAGAGSGAGAGSGAGAGSGAGAGSGAGAGSGAGAGSGAGAGYGAGYGAGVGAGYGAGAGVGYGAGAGAGYGAGAGSGAASGAGAGAGAGAGAGSGAGAGSGAGAGSGAGAGSGAGAGSGAGAGSGAGAGSGAGAGSGAGAGSGAGAGYGAGVGAGYGAGYGGAGAGYGAGAGSGAASGAGAGSGAGAGSGAGAGSGAGAGSGAGAGSGAGAGYGAGAGSGAASGAGAGAGAGAGTGSSGFGPYVNGGYSGYEYAWSSESDFGTGSGAGAGSGAGAGSGAGAGYGAGVGAGYGAGYGAGAGAGYGAGAGSGAASGAGAGSGAGAGSGAGAGSGAGAGSGAGSGAGAGSGAGAGSGAGAGSGAGAGSGAGAGSGAGAGYGAGVGAGYGAGYGAGAGAGYGAGAGSGAASGAGAGSGAGAGAGSGAGAGSGAGAGSGAGAGSGAGAGSGAGAGSGAGSGAGAGSGAGAGYGAGYGAGVGAGYGAGAGVGYGAGAGAGYGAGAGSGAASGAGAGSGSGAGSGAGAGSGAGAGSGAGAGAGSGAGAGSGAGAGSGAGAGYGAGYGAGAGSGAASGAGAGAGAGAGTGSSGFGPYVANGGYSGYEYAWSSESDFGTGSGAGAGSGAGAGSGAGAGYGAGVGAGYGAGYGAGAGAGYGAGAGSGAGSGAGAGSGAGAGSGAGAGSGAGAGSGAGAGSGAGAGSGAGAGSGAGAGYGAGYGAGAGAGYGAGAGVGYGAGAGAGYGAGAGSGAGSGAGAGSGSGAGAGSGSGAGSGAGAGSGAGAGSGAGAGSGAGAGSGAGAGSGAGAGSGAGAGYGAGYGIGVGAGYGAGAGVGYGAGAGAGYGAGAGSGAASGAGAGSGAGAGSGAGAGSGAGAGSGAGAGSGAGAGSGAGAGSGAGAGSGAGAGSGAGAGYGAGAGVGYGAGAGSGAASGAGAGSGAGAGSGAGAGSGAGAGSGAGAGSGAGAGSGAGAGSGAGSGAGAGSGAGAGYGAGYGAGVGAGYGAGAGYGAGYGVGAGAGYGAGAGSGAGSGAGAGSGAGAGSGAGAGSGAGAGSGAGAGSGAGSGAGAGYGAGAGAGYGAGAGAGYGAGAGSGAASGAGAGAGAGSGAGAGSGAGAGSGAGSGAGAGSGAGAGYGAGAGSGAASGAGAGSGAGAGAGAGAGAGSGAGAGSGAGAGYGAGAGSGAASGAGAGAGAGTGSSGFGPYVANGGYSRREGYEYAWSSKSDFETGSGAASGAGAGAGSGAGAGSGAGAGSGAGAGSGAGAGGSVSYGAGRGYGQGAGSAASSVSSASSRSYDYSRRNVRKNCGIPRRQLVVKFRALPCVNC

SEQ ID NO: 8 - protein, 262 aa, Bombyx mori
MKPIFLVLLVATSAYAAPSVTINQYSDNEIPRDIDDGKASSVISRAWDYVDDTDKSIAILNVQEILKDMASQGDYASQASAVAQTAGIIAHLSAGIPGDACAAANVINSYTDGVRSGNFAGFRQSLGPFFGHVGQNLNLINQLVINPGQLRYSVGPALGCAGGGRIYDFEAAWDAILASSDSSFLNEEYCIVKRLYNSRNSQSNNIAAYITAHLLPPVAQVFHQSAGSITDLLRGVGNGNDATGLVANAQRYIAQAASQVHV

SEQ ID NO: 9 - protein, 1186 aa, Bombyx mori
MRFVLCCTLIALAALSVKAFGHHPGNRDTVEVKNRKYNAASSESSYLNKDNDSISAGAHRAKSVEQSQDKSKYTSGPEGVSYSGRSQNYKDSKQAYADYHSDPNGGSASAGQSRDSSLRERNVHYVSDGEAVAASSDARDENRSAQQNAQANWNADGSYGVSADRSGSASSRRRQANYYSDKDITAASKDDSRADSSRRSNAYYNRDSDGSESAGLSDRSASSSKNDNVFVYRTKDSIGGQAKSSRSSHSQESDAYYNSSPDGSYNAGTRDSSISNKKKASSTIYADKDQIRAANDRSSSKQLKQSSAQISSGPEGTSVSSKDRQYSNDKRSKSDAYVGRDGTVAYSNKDSEKTSRQSNTNYADQNSVRSDSAASDQTSKSYDRGYSDKNIVAHSSGSRGSQNQKSSSYRADKDGFSSSTNTEKSKFSSSNSVVETSDGASASRESSAEDTKSSNSNVQSDEKSASQSSSSRSSQESASYSSSSSSSTLSEDSSEVDIDLGNLGWWWNSDNKVQRAAGGATKSGASSSTQATTVSGADDSADSYTWWWNPRRSSSSSSSASSSSSGSNVGGSSQSSGSSTSGSNARGHLGTVSSTGSTSNTDSSSKSAGSRTSGGSSTYGYSSSHRGGSVSSTGSSSNTDSSTKNAGSSTSGGSSTYGYSSSHRGGSVSSTGSSSNTDSSTKSAGSSTSGGSSTYGYSSRHRGGRVSSTGSSSTTDASSNSVGSSTSGGSSTYGYSSNSRDGSVSSTGSSSNTDSNSNSAGSSTSGGSSTYGYSSNSRDGSVSSTGSSSNTDSNSNSAGSSTSGGSSTYGYSSNSRDGSVSSTGSSSNTDASTDLTGSSTSGGSSTYGYSSDSRDGSVSSTGSSSNTDASTDLAGSSTSGGSSTYGYSSDCGDGSVSSTGSSSNTDASTDLAGSSTSGGSSTYGYSSDSRDGSVSSTGSSSNTDASTDLAGSSTSGGSSTYGYSSNSRDGSVSSTGSSSNTDASTDLTGSSTSGGSSTYGYSSSNRDGSVLATGSSSNTDASTTEESTTSAGSSTEGYSSSSHDGSVTSTDGSSTSGGASSSSASTAKSDAASSEDGFWWWNRRKSGSGHKSATVQSSTTDKTSTDSASSTDSTSSTSGASTTTSGSSSTSGGSSTSDASSTSSSVSRSHHSGVNRLLHKPGQGKICLCFENIFDIPYHLRKNIGV

SEQ ID NO: 10 - protein, 900 aa, Bombyx mori
MKIPYVLLFLVGVAVVNALPNPLFGGLVKSLSKKKQIFEDKFENLKENVGEKFENLKENVGEKVENLKENVGEKLENIKEKAGEKFENLKDNVGEKFENLKDNVGDKLEAAKEKAGEIKKKLVDVGEDLKDELTEDKKIKISISKDEGLTLEKEGYKSDYDRNEYEERGSEHQEDNDSDGSYSKGSEYEKYGEEEKYEERRTHDKFSIGKNGISAERTKSKRGERKEVEGEYEKDYERKENNGGSSEYSERERESLEKSKERYGEQSSKSFSLGKSGLKKQDNSKSYSDKEESKLEKEKKYEKKTKINNERQLDEDENERRTVVGRDEQRQDDQSRDDQSRDDQSQDEETGSDDSDKNRGKDTDDKYSETGTNKSSETKTGKRDGSKSGVTVEREKSESNKKSREFENKEAESSTYRDKNRSVNSGSERKSSGKDEEYSEQNSSNKSFNDGDASADYQTKSKKVEKNSARDKKEKEKTDTRNSDGTYKTSEREKEQSSRVNQSKGSNSRDSSESDKSGRKVNKETETYSDKDAQTSESERTQSKDNGGLKEKSSQSKNYGRDEKYSEEKERSSTGKFGSNDSRARSTKAEEEHVRKSQEETHSEQREKTRSDGVTKYNDGDEHFDSDDTEKTKPNGRSPSHKDTEKAKPNDRSSSDKDTEKTFDKNIDNKRPKDGSSSDKNVEQERENYKSESSRNEFENQKSAHSRYEDNGGLKEKSSQSKNYGRDEKYSEEKERSSTGKSGSNDSRARSTKAEEEHVRKSQEETHSEQRGRTRSDGATTSNDNDKQYDSDDKNNSSTKHKKTVMRSEQSDSSQNENSTSESKKFAKTDGSNKYEAESSSHKQQEARKQSNRVVEKSTDGDNEESYRSESSSSSSSSSSSSRSSSSSTYTGSHDDSSEE

SEQ ID NO: 11 - protein, 1271 aa, Bombyx mori
MNCKVALFLIVAIVAVQALPCQESRPRRCGYRYGCGGGRGRGSGVRRLDSGADDNQGRSCLVGGSAESNDEDSDDRLSVINNTEGHATSSSFDEQSSSARQSSSSYQSQSYNKDSSSTNESSDGGSGSGRTGSAGENGENSDDSSGATKGNSSKSSSSSQGQSASSSSSDEKSSQSSSNSSNNSKSSSQSSSSQNSSGSKGSGSEESSNGGSGSGRTGSAGGTDEDSDDSSGATKGNSSKSSSSSQGQSASSSSSDENSSQSSSNSSNNSKSSSQSSSGQNSSGSKGSGSEESSNGGSGSGRNGSVGGTDEDSDDSSGATKGNSSKSSSSSQGQSASSSSSDEKSSQSSSNSSNNSKSSSQSSSGQNSSGSKGSGSEESSNGGSGSGRNGSAGGTDEDSDDSSGATKGNSSKSSSSSQGQSASSSSSDEKSSQSSSNSSNNSKSSSQSSSGQNSSGSKGSGSEESSNGGSGSGRNGSAGGTDEDSDDSSGATKGNSSKSSSSSQGQSASSSSSDEKSSQSSSNSSNNSKSSSQSSSGQNSSGSKGSGSEESSNGGSGSGRTGSAGETDEDSDDSSGATKGNSSKSSSSSQGKSASSSSSDEKSSQSSSNSSNNSKSSSQSSSSNNSSGSKGSGSEESSNGGSGSGRTGSAGGSDEDSDDSSGATKGNSSKSSSSSQGQSASSSSSDEKSSQSNSNSSNNSKSSSQSSSSNNSSGSKGSGSEESSNGGSGSGRTGSAGGTDEDSDDSSGATKGNSSKSSSSSQGKSASSSSSDEKSSQSSSNSSNNSKSSSQSSSSKNSSGSKGSGSEESSNGGSGSGRTGSAGGTDEDSDDSSGATKGNSSKSSSSSQGKSASSSSSDEKSSQSNSNSSNNSKSSSQSSSSKNSSGSKGSGSEESSNGGSGSGRTGSAGGTDEDSDDSSGATKGNSSKSSSSSQGKSASSSSSNEKSSQSSSNSSNNSKSSSQSSSSKNSSGSKGSGSSESGDKKSSSRGSSGDNSDDDQTDSARSNSKRSTSSDASTKKSSSRKSSNHRSSRSQQAHSSSSKQAQSSSSQQAQNSRSQQAHSSRSQQAHSSSSKQAQSSSSKQAQSSSSKQAQSSSSKQAQSSSSQQAQSSRSQQAHSSRSQQAHSSSSKQAQSSSSKQAQSSSSKQAQSSSSKQAQSSSSQQAQSSRSQQAHSSRSETDSKSSNSGGHSNHSSRTEQKSSAKAISSSEQSQNFSSSSQKSAEAADGSESTQSASEYSSSQSKASSSFSASSASESSSLSSDVNFEEKTD

SEQ ID NO: 12 - protein, 748 aa, Nephila clavipes
QGAGAAAAAAGGAGQGGYGGLGGQGAGQGGYGGLGGQGAGQGAGAAAAAAAGGAGQGGYGGLGSQGAGRGGQGAGAAAAAAGGAGQGGYGGLGSQGAGRGGLGGQGAGAAAAAAAGGAGQGGYGGLGNQGAGRGGQGAAAAAAGGAGQGGYGGLGSQGAGRGGLGGQGAGAAAAAAGGAGQGGYGGLGGQGAGQGGYGGLGSQGAGRGGLGGQGAGAAAAAAAGGAGQGGLGGQGAGQGAGASAAAAGGAGQGGYGGLGSQGAGRGGEGAGAAAAAAGGAGQGGYGGLGGQGAGQGGYGGLGSQGAGRGGLGGQGAGAAAAGGAGQGGLGGQGAGQGAGAAAAAAGGAGQGGYGGLGSQGAGRGGLGGQGAGAVAAAAAGGAGQGGYGGLGSQGAGRGGQGAGAAAAAAGGAGQRGYGGLGNQGAGRGGLGGQGAGAAAAAAAGGAGQGGYGGLGNQGAGRGGQGAAAAAGGAGQGGYGGLGSQGAGRGGQGAGAAAAAAVGAGQEGIRGQGAGQGGYGGLGSQGSGRGGLGGQGAGAAAAAAGGAGQGGLGGQGAGQGAGAAAAAAGGVRQGGYGGLGSQGAGRGGQGAGAAAAAAGGAGQGGYGGLGGQGVGRGGLGGQGAGAAAAGGAGQGGYGGVGSGASAASAAASRLSSPQASSRVSSAVSNLVASGPTNSAALSSTISNVVSQIGASNPGLSGCDVLIQALLEVVSALIQILGSSSIGQVNYGSAGQATQIVGQSVYQALG

SEQ ID NO: 13 - protein, 627 aa, Nephila clavipes
PGGYGPGQQGPGGYGPGQQGPSGPGSAAAAAAAAAAGPGGYGPGQQGPGGYGPGQQGPGRYGPGQQGPSGPGSAAAAAAGSGQQGPGGYGPRQQGPGGYGQGQQGPSGPGSAAAASAAASAESGQQGPGGYGPGQQGPGGYGPGQQGPGGYGPGQQGPSGPGSAAAAAAAASGPGQQGPGGYGPGQQGPGGYGPGQQGPSGPGSAAAAAAAASGPGQQGPGGYGPGQQGPGGYGPGQQGLSGPGSAAAAAAAGPGQQGPGGYGPGQQGPSGPGSAAAAAAAAAGPGGYGPGQQGPGGYGPGQQGPSGAGSAAAAAAAGPGQQGLGGYGPGQQGPGGYGPGQQGPGGYGPGSASAAAAAAGPGQQGPGGYGPGQQGPSGPGSASAAAAAAAAGPGGYGPGQQGPGGYAPGQQGPSGPGSASAAAAAAAAGPGGYGPGQQGPGGYAPGQQGPSGPGSAAAAAAAAAGPGGYGPAQQGPSGPGIAASAASAGPGGYGPAQQGPAGYGPGSAVAASAGAGSAGYGPGSQASAAASRLASPDSGARVASAVSNLVSSGPTSSAALSSVISNAVSQIGASNPGLSGCDVLIQALLEIVSACVTILSSSSIGQVNYGAASQFAQVVGQSVLSAF